European Patent Application EP 4 600 370 A1, published August 13, 2025. Title: NudE.1 as a decapping enzyme for cofactor- and “canonically"-capped RNA species. Applicant: Max-Planck-Gesellschaft zur Förderung der Wissenschaften e.V. The sequence listing filed with the application follows.

SEQUENCE LISTING (28 sequences)

SEQ ID NO: 1 - DNA, 43 bp, synthetic construct
  source 1..43: mol_type = other DNA; note = NudE.1 fwd NcoI
atcgacccatgggacaggaaattaaaatgaaaacattatcagc

SEQ ID NO: 2 - DNA, 60 bp, synthetic construct
  source 1..60: mol_type = other DNA; note = NudE.1 rev XhoI
gtgctcgaggccctgaaaataaagattctcaccaaagaggttgttcattattcggtaaag

SEQ ID NO: 3 - DNA, 33 bp, synthetic construct
  source 1..33: mol_type = other DNA; note = NudE.1 E64,65Q fwd
cgaagagaatgtttacaacagactggttttagc

SEQ ID NO: 4 - DNA, 24 bp, synthetic construct
  source 1..24: mol_type = other DNA; note = NudE.1 E64,65Q rev
tgctgcatctaatgcgcttaaatc

SEQ ID NO: 5 - DNA, 76 bp, synthetic construct
  source 1..76: mol_type = other DNA; note = Fwd ultramer IVT Qbeta
taatacgactcactattatcttgatactacctttagttcgtttaaacacgttcttgatagtatctttttattaacc

SEQ ID NO: 6 - DNA, 71 bp, synthetic construct
  source 1..71: mol_type = other DNA; note = Rev ultramer IVT Qbeta
catgatcaaattgacccaaagtttcaacgctttacgcgttgggttaataaaaagatactatcaagaacgtg

SEQ ID NO: 7 - DNA, 36 bp, synthetic construct
  source 1..36: mol_type = other DNA; note = Fwd primer IVT Qbeta
taatacgactcactattatcttgatactacctttag

SEQ ID NO: 8 - DNA, 38 bp, synthetic construct
  source 1..38: mol_type = other DNA; note = Rev primer IVT Qbeta
catgatcaaattgacccaaagtttcaacgctttacgcg

SEQ ID NO: 9 - DNA, 82 bp, synthetic construct
  source 1..82: mol_type = other DNA; note = Fwd ultramer IVT RNAI
taatacgactcactattacagtatttggtatctgcgctctgctgaagccagttaccttcggaaaaagagttggtagctcttg

SEQ ID NO: 10 - DNA, 82 bp, synthetic construct
  source 1..82: mol_type = other DNA; note = Rev ultramer IVT RNAI
aacaaaaaaaccaccgctaccagcggtggtttgtttgccggatcaagagctaccaactctttttccgaaggtaactggcttc

SEQ ID NO: 11 - DNA, 21 bp, synthetic construct
  source 1..21: mol_type = other DNA; note = Fwd primer IVT RNAI
taatacgactcactattacag

SEQ ID NO: 12 - DNA, 21 bp, synthetic construct
  source 1..21: mol_type = other DNA; note = Rev primer IVT RNAI
aacaaaaaaaccaccgctacc

SEQ ID NO: 13 - RNA, 100 nt, synthetic construct
  source 1..100: mol_type = other RNA; note = Qbeta-RNA
atcttgatactacctttagttcgtttaaacacgttcttgatagtatctttttattaacccaacgcgtaaagcgttgaaactttgggtcaatttgatcatg

SEQ ID NO: 14 - RNA, 108 nt, synthetic construct
  source 1..108: mol_type = other RNA; note = RNAI
acagtatttggtatctgcgctctgctgaagccagttaccttcggaaaaagagttggtagctcttgatccggcaaacaaaccaccgctggtagcggtggtttttttgtt

SEQ ID NO: 15 - RNA, 10 nt, synthetic construct
  source 1..10: mol_type = other RNA; note = 10mer-Cy5
acagtatttg

SEQ ID NO: 16 - RNA, 40 nt, synthetic construct
  source 1..40: mol_type = other RNA; note = DNA-40mer-Cy5
acagtatttggtatctgcgctctgctgaagccagttacct

SEQ ID NO: 17 - DNA, 507 bp, synthetic construct
  source 1..507: mol_type = other DNA; note = pET28-NudE.1 WT
atgggacaggaaattaaaatgaaaacattatcagctggtattatctttatgacagaagataaagatttatttatgggtcgggttactggttctcgtaagactggaatgatggcacatcgttgggatattccaaagggccgtgtagaaaattctgatttaagcgcattagatgcagcacgaagagaatgtttagaagagactggttttagcaattataatccagaccttctagaagacctaggtgtatttaaatattctagtaataaagacctacagttattttattacacgattccagtagagcatgagatgttcagaaattgccgttgcgagtcttattttgaaaataaagatggcgttatgattccagagatggacgcttttgctcttattcctcgtactcagtggcaatatgtgatgggtccttcactttaccgaataatgaacaacctctttggtgagaatctttattttcagggcctcgagcaccaccaccaccaccactga

SEQ ID NO: 18 - DNA, 507 bp, synthetic construct
  source 1..507: mol_type = other DNA; note = pET28-NudE.1 M1
atgggacaggaaattaaaatgaaaacattatcagctggtattatctttatgacagaagataaagatttatttatgggtcgggttactggttctcgtaagactggaatgatggcacatcgttgggatattccaaagggccgtgtagaaaattctgatttaagcgcattagatgcagcacgaagagaatgtttacaacagactggttttagcaattataatccagaccttctagaagacctaggtgtatttaaatattctagtaataaagacctacagttattttattacacgattccagtagagcatgagatgttcagaaattgccgttgcgagtcttattttgaaaataaagatggcgttatgattccagagatggacgcttttgctcttattcctcgtactcagtggcaatatgtgatgggtccttcactttaccgaataatgaacaacctctttggtgagaatctttattttcagggcctcgagcaccaccaccaccaccactga

SEQ ID NO: 19 - DNA, 822 bp, synthetic construct
  source 1..822: mol_type = other DNA; note = pET28-NudC WT
atggatcgtataattgaaaaattagatcacggctggtgggtcgtcagccatgaacaaaaattatggttgccgaagggagaattgccatatggcgaagcggcaaatttcgatcttgtgggtcagcgcgcactacaaatcggcgaatggcagggggaacctgtttggttagtacaacagcagcggcgtcacgatatggggtcggtacgtcaggtcattgatctcgatgttgggctgtttcaactggccggacgaggcgtacaactggcggagttttaccgatcgcataaatactgtggttactgcgggcatgaaatgtatccgagcaaaaccgaatgggcgatgctgtgcagccattgccgtgagcgttactacccgcaaatcgccccctgcattattgttgccatccgtcgcgatgattcgatcctcctcgcccagcatacccgccatcgtaacggtgtccatacagtacttgccggattcgtcgaagtgggcgaaaccctcgagcaggcagtcgcgcgggaagtgatggaagagagcggaattaaagttaaaaacttgcgttacgtgacttctcagccgtggccgtttcctcagtctttaatgaccgcgtttatggcggaatatgacagcggcgacatcgtgatcgacccgaaagaattgctcgaggcgaactggtatcgctatgacgatttgccgttactcccgccgcccggcaccgtagcgcgccgtctgatagaagatacggtggcgatgtgtcgggcagagtatgagctggtgccgcgcggcagcgcggccgcactcgagcaccaccaccaccaccac

SEQ ID NO: 20 - DNA, 822 bp, synthetic construct
  source 1..822: mol_type = other DNA; note = pET28-NudC M1
atggatcgtataattgaaaaattagatcacggctggtgggtcgtcagccatgaacaaaaattatggttgccgaagggagaattgccatatggcgaagcggcaaatttcgatcttgtgggtcagcgcgcactacaaatcggcgaatggcagggggaacctgtttggttagtacaacagcagcggcgtcacgatatggggtcggtacgtcaggtcattgatctcgatgttgggctgtttcaactggccggacgaggcgtacaactggcggagttttaccgatcgcataaatactgtggttactgcgggcatgaaatgtatccgagcaaaaccgaatgggcgatgctgtgcagccattgccgtgagcgttactacccgcaaatcgccccctgcattattgttgccatccgtcgcgatgattcgatcctcctcgcccagcatacccgccatcgtaacggtgtccatacagtacttgccggattcgtcgaagtgggcgaaaccctcgagcaggcagtcgcgcgggaagtgatggaacagagcggaattaaagttaaaaacttgcgttacgtgacttctcagccgtggccgtttcctcagtctttaatgaccgcgtttatggcggaatatgacagcggcgacatcgtgatcgacccgaaagaattgctcgaggcgaactggtatcgctatgacgatttgccgttactcccgccgcccggcaccgtagcgcgccgtctgatagaagatacggtggcgatgtgtcgggcagagtatgagctggtgccgcgcggcagcgcggccgcactcgagcaccaccaccaccaccac

SEQ ID NO: 21 - protein, 168 aa, synthetic construct
  source 1..168: note = pET28-NudE.1 WT
MGQEIKMKTLSAGIIFMTEDKDLFMGRVTGSRKTGMMAHRWDIPKGRVENSDLSALDAARRECLEETGFSNYNPDLLEDLGVFKYSSNKDLQLFYYTIPVEHEMFRNCRCESYFENKDGVMIPEMDAFALIPRTQWQYVMGPSLYRIMNNLFGENLYFQGLEHHHHHH

SEQ ID NO: 22 - protein, 168 aa, synthetic construct
  source 1..168: note = pET28-NudE.1 M1
MGQEIKMKTLSAGIIFMTEDKDLFMGRVTGSRKTGMMAHRWDIPKGRVENSDLSALDAARRECLQQTGFSNYNPDLLEDLGVFKYSSNKDLQLFYYTIPVEHEMFRNCRCESYFENKDGVMIPEMDAFALIPRTQWQYVMGPSLYRIMNNLFGENLYFQGLEHHHHHH

SEQ ID NO: 23 - protein, 274 aa, synthetic construct
  source 1..274: note = pET28-NudC WT
MDRIIEKLDHGWWVVSHEQKLWLPKGELPYGEAANFDLVGQRALQIGEWQGEPVWLVQQQRRHDMGSVRQVIDLDVGLFQLAGRGVQLAEFYRSHKYCGYCGHEMYPSKTEWAMLCSHCRERYYPQIAPCIIVAIRRDDSILLAQHTRHRNGVHTVLAGFVEVGETLEQAVAREVMEESGIKVKNLRYVTSQPWPFPQSLMTAFMAEYDSGDIVIDPKELLEANWYRYDDLPLLPPPGTVARRLIEDTVAMCRAEYELVPRGSAAALEHHHHHH

SEQ ID NO: 24 - protein, 274 aa, synthetic construct
  source 1..274: note = pET28-NudC M1
MDRIIEKLDHGWWVVSHEQKLWLPKGELPYGEAANFDLVGQRALQIGEWQGEPVWLVQQQRRHDMGSVRQVIDLDVGLFQLAGRGVQLAEFYRSHKYCGYCGHEMYPSKTEWAMLCSHCRERYYPQIAPCIIVAIRRDDSILLAQHTRHRNGVHTVLAGFVEVGETLEQAVAREVMEQSGIKVKNLRYVTSQPWPFPQSLMTAFMAEYDSGDIVIDPKELLEANWYRYDDLPLLPPPGTVARRLIEDTVAMCRAEYELVPRGSAAALEHHHHHH

SEQ ID NO: 25 - protein, 24 aa, synthetic construct
  source 1..24: note = Nudix hydrolase shared structural consensus motif
  VARIANT 13: note = F, I, L, or V
  VARIANT 24: note = F, I, L, or V
GXXXXXEXXXXXXAXREXXEEXGX

SEQ ID NO: 26 - protein, 24 aa, synthetic construct
  source 1..24: note = NudE.1 shared structural motif
GRVENSDLSALDAARRECLEETGF

SEQ ID NO: 27 - protein, 207 aa, Escherichia virus T4
  source 1..207: note = ART ModB from Escherichia virus T4
MIINLADVEQLSIKAESVDFQYDMYKKVCEKFTDFEQSVLWQCMEAKKNEALHKHLNEIIKKHLTKSPYQLYRGISKSTKELIKDLQVGEVFSTNRVDSFTTSLHTACSFSYAEYFTETILRLKTDKAFNYSDHISDIILSSPNTEFKYTYEDTDGLDSERTDNLMMIVREQEWMIPIGKYKITSISKEKLHDSFGTFKVYDIEVVE

SEQ ID NO: 28 - protein, 222 aa, synthetic construct
  source 1..222: note = cloned ModB
MGIINLADVEQLSIKAESVDFQYDMYKKVCEKFTDFEQSVLWQCMEAKKNEALHKHLNEIIKKHLTKSPYQLYRGISKSTKELIKDLQVGEVFSTNRVDSFTTSLHTACSFSYAEYFTETILRLKTDKAFNYSDHISDIILSSPNTEFKYTYEDTDGLDSERTDNLMMIVREQEWMIPIGKYKITSISKEKLHDSFGTFKVYDIEVVELVPRGSLEHHHHHH